European Patent Specification EP 3 277 622 B1, published August 2, 2023. Title: Nanocomposite material. Applicant: James Hutton Institute CELLUCOMP LIMITED TALIANSKY, Michael LOVE, Andrew WHALE, Eric Hepworth, David. Application GB1505767.2. The sequence listing filed with the application follows.

SEQUENCE LISTING (4 sequences)

SEQ ID NO: 1 - DNA, 44 bp, Artificial Sequence
  MIP3 primer - forward
ccggctctgaatctgattcttctgattctgattctaagtctgta

SEQ ID NO: 2 - DNA, 40 bp, Artificial Sequence
  MIP3 primer - reverse
tacagacttagaatcagaatcagaagaatcagattcagag

SEQ ID NO: 3 - DNA, 38 bp, Artificial Sequence
  MBP primer - forward
ccggctctgaaaagctttggtggggagcttctcttgta

SEQ ID NO: 4 - DNA, 35 bp, Artificial Sequence
  MBP primer - reverse
tacaaagagaagctccccaccaaagcttttcagag